European Patent Application EP 4 732 836 A1, published April 29, 2026. Title: Use of AG5 compound in fatty liver diseases. Applicant: CONSEJO SUPERIOR DE INVESTIGACIONES CIENTIFICAS. Application EP. The sequence listing filed with the application follows.

SEQUENCE LISTING (12 sequences)

SEQ ID NO: 1 - DNA, 23 bp, synthetic construct
  source 1..23: mol_type = other DNA; organism (original language) = constructo sintetico
gcgattccttcactgatacactg

SEQ ID NO: 2 - DNA, 23 bp, synthetic construct
  source 1..23: mol_type = other DNA; organism (original language) = constructo sintetico
gagtgggagtggtcttccattac

SEQ ID NO: 3 - DNA, 25 bp, synthetic construct
  source 1..25: mol_type = other DNA; organism (original language) = constructo sintetico
aagaagcagcaaaatgtacctgaag

SEQ ID NO: 4 - DNA, 23 bp, synthetic construct
  source 1..23: mol_type = other DNA; organism (original language) = constructo sintetico
cctgattggtatgggtttcactc

SEQ ID NO: 5 - DNA, 22 bp, synthetic construct
  source 1..22: mol_type = other DNA; organism (original language) = constructo sintetico
tcagtgtgaatggggatgtgat

SEQ ID NO: 6 - DNA, 22 bp, synthetic construct
  source 1..22: mol_type = other DNA; organism (original language) = constructo sintetico
tctgcacatgtaccaggacacc

SEQ ID NO: 7 - DNA, 21 bp, synthetic construct
  source 1..21: mol_type = other DNA; organism (original language) = constructo sintetico
ccaacaccagcatccagttca

SEQ ID NO: 8 - DNA, 21 bp, synthetic construct
  source 1..21: mol_type = other DNA; organism (original language) = constructo sintetico
atccctgcttgcacatctctc

SEQ ID NO: 9 - DNA, 21 bp, synthetic construct
  source 1..21: mol_type = other DNA; organism (original language) = constructo sintetico
aagctgaaggacctgtctagg

SEQ ID NO: 10 - DNA, 21 bp, synthetic construct
  source 1..21: mol_type = other DNA; organism (original language) = constructo sintetico
cggagtgaatctgggttgatg

SEQ ID NO: 11 - DNA, 22 bp, synthetic construct
  source 1..22: mol_type = other DNA; organism (original language) = constructo sintetico
ttttggtgacgacttgaactgc

SEQ ID NO: 12 - DNA, 22 bp, synthetic construct
  source 1..22: mol_type = other DNA; organism (original language) = constructo sintetico
ccatcttgtccaccacctcttc